European Patent Application EP 4 745 250 A1, published May 20, 2026. Title: Detection Chip for African Swine Fever Virus and Application Thereof. Applicant: Sunplus Technology Co. Ltd. Application EA. The sequence listing filed with the application follows.

SEQUENCE LISTING (4 sequences)

SEQ ID NO: 1 - DNA, 25 bp, synthetic construct
  source 1..25: mol_type = other DNA
ccacgggaggaataccaacccagtg

SEQ ID NO: 2 - DNA, 20 bp, synthetic construct
  source 1..20: mol_type = other DNA
caagtgtaggcaagccagtc

SEQ ID NO: 3 - DNA, 19 bp, synthetic construct
  source 1..19: mol_type = other DNA
ccatgactagtctgtccgt

SEQ ID NO: 4 - DNA, 20 bp, synthetic construct
  source 1..20: mol_type = other DNA
acgggcagaccggcaacaaa